European Patent Application EP 4 692 104 A1, published February 11, 2026. Title: CONJUGATE OF ANTIBODY AND FUNCTIONAL SUBSTANCE OR SALT OF SAID CONJUGATE, AND ANTIBODY INTERMEDIATE HAVING THIOL GROUP OR SALT OF SAID ANTIBODY INTERMEDIATE. Applicant: AJINOMOTO CO., INC. Application EP EP24784960.7, filed April 4, 2024. The sequence listing filed with the application follows.

SEQUENCE LISTING (15 sequences)

SEQ ID NO: 1 - protein, 17 aa, synthetic construct
RGNCAYHKGQLVWCTYH

SEQ ID NO: 2 - protein, 34 aa, synthetic construct
FNMQCQRRFYEALHDPNLNEEQRNARIRSIKEEC

SEQ ID NO: 3 - protein, 17 aa, synthetic construct
RGNCAYHKGQIIWCTYH

SEQ ID NO: 4 - protein, 4 aa, synthetic construct
GGPG

SEQ ID NO: 5 - protein, 4 aa, synthetic construct
GGFG

SEQ ID NO: 6 - protein, 4 aa, synthetic construct
DDVD

SEQ ID NO: 7 - protein, 4 aa, synthetic construct
EEVC

SEQ ID NO: 8 - protein, 6 aa, synthetic construct
EEEEVC

SEQ ID NO: 9 - protein, 5 aa, synthetic construct
EGGFG

SEQ ID NO: 10 - protein, 4 aa, synthetic construct
EEFK

SEQ ID NO: 11 - protein, 4 aa, synthetic construct
EEVK

SEQ ID NO: 12 - protein, 4 aa, synthetic construct
EEAK

SEQ ID NO: 13 - protein, 5 aa, synthetic construct
EEVLK

SEQ ID NO: 14 - protein, 5 aa, synthetic construct
EDDVD

SEQ ID NO: 15 - protein, 4 aa, synthetic construct
EEGC